European Patent Specification EP 3 464 572 B1, published July 26, 2023. Title: VARIANTS OF ACETYLSEROTONIN 0-METHYLTRANSFERASE AND USES THEREOF. Applicant: Danmarks Tekniske Universitet. The sequence listing filed with the application follows.

SEQUENCE LISTING (20 sequences)

SEQ ID NO: 1 - protein, 345 aa, Homo sapiens
MGSSEDQAYRLLNDYANGFMVSQVLFAACELGVFDLLAEAPGPLDVAAVAAGVRASAHGTELLLDICVSLKLLKVETRGGKAFYRNTELSSDYLTTVSPTSQCSMLKYMGRTSYRCWGHLADAVREGRNQYLETFGVPAEELFTAIYRSEGERLQFMQALQEVWSVNGRSVLTAFDLSVFPLMCDLGGGAGALAKECMSLYPGCKITVFDIPEVVWTAKQHFSFQEEEQIDFQEGDFFKDPLPEADLYILARVLHDWADGKCSHLLERIYHTCKPGGGILVIESLLDEDRRGPLLTQLYSLNMLVQTEGQERTPTHYHMLLSSAGFRDFQFKKTGAIYDAILARK

SEQ ID NO: 2 - protein, 361 aa, Ocimicum basilicum
MSSTANNPQINSDEEENFLFAMQLASASVLPMVLKSAIELDLLELIKKAGAGAFVSPAELAAQLLTTNAEAHVMLDRILRLLTSYAILECRLKTLPDGGVQRLYGLAPVCKFLTKNEDGVSMAPLALMNQDKVLMESWYHLKDAVLDGGIPFNKAYGMTAFEYHGTDPRFNKVFNQGMSNHSTITMKKILETYTGFDGLKTVVDVGGGTGATLNMIISKYPSIKGINFDLPHVVEDAPSYPGVEHVGGDMFVSVPKGDAIFMKWICHDWSDAHCVKFLKKCYEALPENGKVILAECVLPEAPDTGLATKNVVHIDVIMLAHNPGGKERTEKEFQVLAKASGFKQFNKVCCAYNSWIMELLK

SEQ ID NO: 3 - protein, 345 aa, Bos taurus
MCSQEGEGYSLLKEYANGFMVSQVLFAACELGVFELLAEALEPLDSAAVSSHLGSSPQGTELLLNTCVSLKLLQADVRGGKAVYANTELASTYLVRGSPRSQRDMLLYAGRTAYVCWRHLAEAVREGRNQYLKAFGIPSEELFSAIYRSEDERLQFMQGLQDVWRLEGATVLAAFDLSPFPLICDLGGGSGALAKACVSLYPGCRAIVFDIPGVVQIAKRHFSASEDERISFHEGDFFKDALPEADLYILARVLHDWTDAKCSHLLQRVYRACRTGGGILVIESLLDTDGRGPLTTLLYSLNMLVQTEGRERTPAEYRALLGPAGFRDVRCRRTGGTYDAVLARK

SEQ ID NO: 4 - protein, 335 aa, Takifugu rubripes
MFLIAHLPLPQVVFSSCELGVFDLLLGAERPLSAEEISRALGTSVDGTERLLAACSGLQLLNIHQDNGRCLYSNTDQASVYLTRSSPVSLSQSIQYSSRTIYLCWHYLTDAVREGRNQYEKAFGVDAQDLFQALYRSDEEMVKFMQLMNSIWNICGKDVVTAFDLSPFKTICDLGGCSGALAKQCTSAYPECTVTIFDLPKVVRTSRENFFTEANQRIGFCEGDFFKDPLPEADLYVLARILHDWTDQRCLELLRRVHGACRPGGSVLLVEALLYEDGSGPLTAQLYSLNMLVQTEGRERSAAQYAALLTAAGFSNVQHRFTGKIYDAVLARKEA

SEQ ID NO: 5 - protein, 345 aa, Macaca mulatta
MGSSGDDGYRLLNEYTNGFMVSQVLFAACELGVFDLLAEAPGPLDVAAVAAGVEASSHGTELLLDTCVSLKLLKVETRAGKAFYQNTELSSAYLTRVSPTSQCNLLKYMGRTSYGCWGHLADAVREGKNQYLQTFGVPAEDLFKAIYRSEGERLQFMQALQEVWSVNGRSVLTAFDLSGFPLMCDLGGGPGALAKECLSLYPGCKVTVFDVPEVVRTAKQHFSFPEEEEIHLQEGDFFKDPLPEADLYILARILHDWADGKCSHLLERVYHTCKPGGGILVIESLLDEDRRGPLLTQLYSLNMLVQTEGQERTPTHYHMLLSSAGFRDFQFKKTGAIYDAILVRK

SEQ ID NO: 6 - protein, 345 aa, Elephantulus edwardii
MEGPGDRAFRLLNEYSSGFMVSQVLFAACELGVFDLLAQAPEPLDTAELATRLGTSLHGTELLLDVCASLELLTVETKRNRAVYQNTDLSTTFLVRTSPTCQLHMLLYLSRTTYLCWGHLAAAVREGKNQYKRAFGVPSEQLFTAIYRSEAERLLFMRGLAEIWSVHGVGVMTAFDLSAFSVICDLGGASGALARVCASLYPDSSVLVLEVPEVVRAARSLFLSTVEAPVSFREGDFFKDPLPEADLYILARVLHDWTDEKCSELLAKIHHTCKPGGGILVVESVLEEDRRGPLTTQLYSLNMLVQTEGRERTPAEYRSLICSAGFQDFQLKKTGKIYDVILARK

SEQ ID NO: 7 - protein, 364 aa, Oryza sativa
MAQNVQENEQVMSTEDLLQAQIELYHHCLAFIKSMALRAATDLRIPDAIHCNGGAATLTDLAAHVGLHPTKLSHLRRLMRVLTLSGIFTVHDGDGEATYTLTRVSRLLLSDGVERTHGLSQMVRVFVNPVAVASQFSLHEWFTVEKAAAVSLFEVAHGCTRWEMIANDSKDGSMFNAGMVEDSSVAMDIILRKSSNVFRGINSLVDVGGGYGAVAAAVVRAFPDIKCTVLDLPHIVAKAPSNNNIQFVGGDLFEFIPAADVVLLKCILHCWQHDDCVKIMRRCKEAISARDAGGKVILIEVVVGIGSNETVPKEMQLLFDVFMMYTDGIEREEHEWKKIFLEAGFSDYKIIPVLGVRSIIEVYP

SEQ ID NO: 8 - protein, 432 aa, Rattus norvegicus
MAPGREGELDRDFRVLMSLAHGFMVSQVLFAALDLGIFDLAAQGPVAAEAVAQTGGWSPRGTQLLMDACTRLGLLRGAGDGSYTNSALSSTFLVSGSPQSQRCMLLYLAGTTYGCWAHLAAGVREGRNQYSRAVGISAEDPFSAIYRSEPERLLFMRGLQETWSLCGGRVLTAFDLSRFRVICDLGGGSGALAQEAARLYPGSSVCVFDLPDVIAAARTHFLSPGARPSVRFVAGDFFRSRLPRADLFILARVLHDWADGACVELLGRLHRACRPGGALLLVEAVLAKGGAGPLRSLLLSLNMMLQAEGWERQASDYRNLATRAGFPRLQLRRPGGPYHAMLARRGPRPGIITGVGSNTTGTGSFVTGIRRDVPGARSDAAGTGSGTGNTGSGIMLQGETLESEVSAPQAGSDVGGAGNEPRSGTLKQGDWK

SEQ ID NO: 9 - protein, 346 aa, Gallus gallus
MDSTEDLDYPQIIFQYSNGFLVSKVMFTACELGVFDLLLQSGRPLSLDVIAARLGTSIMGMERLLDACVGLKLLAVELRREGAFYRNTEISNIYLTKSSPKSQYHIMMYYSNTVYLCWHYLTDAVREGRNQYERAFGISSKDLFGARYRSEEEMLKFLAGQNSIWSICGRDVLTAFDLSPFTQIYDLGGGGGALAQECVFLYPNCTVTIYDLPKVVQVAKERLVPPEERRIAFHEGDFFKDSIPEADLYILSKILHDWDDKKCRQLLAEVYKACRPGGGVLLVESLLSEDRSGPVETQLYSLNMLVQTEGKERTAVEYSELLGAAGFREVQVRRTGKLYDAVLGRK

SEQ ID NO: 10 - protein, 341 aa, Chromobacterium violaceum
MGYAAPQARQSDKKIFDIYFGFLHSYALLFADEVGLFDLLRCEALTLDQVSMATSLPFRSSQALLSLCASLGLLEKRGERFALSALAEGFLVREAETSFCGVLASARGQAAAFSYDFFKASLLKGESQLFGGRDLFDNNAQDSEHCEIFTRAMHSKSKGPAQAWVEKIDLSAHACLLDVGGGSGVHAISALARWPNLNAVVFDLPPVCAIADTFIERYQMMARAQTHGGDIWYTDYPFADAHFYSDIFHDWPLERCRFLARKSFDALPSGGRIILHEMLFNTQKTGPRNVAAYNANMLLWTQGQQLSEPEAADLLQAAGFVEILAFPTGYGDWSLVTGVKP

SEQ ID NO: 11 - protein, 338 aa, Desulfotomaculum kuznetsovii DSM 6115
MYTGETRFSPSGWYIMDICRGHWAAQVLFTAVDLGLFDILARGAQTPARVAAALGTHPEATARLLVALEGLGLVKREGEFYRNAPLAGRHLVRGGDAYLGHAVHHFANLAEGWSRLGEAVRTGRPVGFEAVERANYEERLRDYILAMGDQARLKADRLAAALDLSGCERILDLGGGPGVHTVALLKKEPRARATILDLAPTLKITRELIEAAGMMERVELCAGDFTRDELGEGVYDLVLASNVVHIYDAATNRQIMDRVFRALRPGGQVVIHDYVLAEEPSLEAALFDLNMLVGTLTGRVYGVQEMGSWLEDAGFVDVTYHPLTPGSGLLKGRKWNDK

SEQ ID NO: 12 - protein, 266 aa, Xenopus (Silurana) tropicalis
MKNNEAFFSNTDVSNMYLVKSSPRSFYQMMMYYSKTIYMCWHFLPDAIREGKRQYERAFGITSEDIFKDLYRSEEETVSFMHHMESIWHICGKDVLAAFDLSSFKEICDIGGCSGGLAKHFLSLYPSSSVTIMDLPEVVQMAKKHFITDGDIVFLEDFFNDPLPESDLYILARIIHDWTEDKCLRLLNKIYKSCRPGGGVLLVEALLNEDRSGPLSSQMFSLNMLLQTEGKERSASEYHKLLADSGFREIQVKATGKFYDAVLGKK

SEQ ID NO: 13 - protein, 341 aa, Pseudomonas fluorescens
MDSTVHTEHHSDKQIFDIYFGFINTYTLFFADEVKLFDLLEGKALRLGEIGSALELAPRAAQALVAMCTSQGLLEKSGECYGLTSLAQAFLTRKSETSFSGVLQSARHKEDAFSYAFFKESMLSGESGLFGETDLFENNAQDQLHSEIFTKAMHSKSKGPARAWSGRIDLSGYTCLLDVGGGSGVHSICALEKWPELNAVIFDLPYVCDIADTYVEQYRMAGRITTHKGDIWASEYPAADVHLYSDIFHDWPLDKCLFLAKKSFDALPSGGRIILHEMFFNKDKTGPHNVAAYNANMLLWTQGQQLSETEIRELLTIAGFRDITVSRTQYGDWSLATGIKY

SEQ ID NO: 14 - protein, 339 aa, Candidatus Solibacter usitatus
MTPNLPDASPVLDLIEAFRRSKTMFTALSMGVFDTLHEAPSNAETLAAKLGANAGALARLLDGCAALQLLQKRDGLYENAPLSETYLYSGSPHSMSGYVRYSEQALYPMWGNLADAVREGTPRWSQNFGIDGPIFSAFFRTPEAMRDFLMGMHGFGMLTSPKVAAAFDLSRFRRLVDLGGATGHLTIAACELYPEMRGVVFDLPQAAGMARELVERSAASARVEIVSGDFFADELPEADLYYTGRILHDWSEEKIDRLLARIVQRLPSGGALLIGEKLLAEDGVGPVPANMQSLNMLVVTEGRERSLGEYRGLLMRAGFASVEGRHTGVALDAILAIKA

SEQ ID NO: 15 - protein, 221 aa, Fenneropenaeus chinensis
MSSLKSYDNTDPLVQYCVNHSLRLTDVQKRLNDATLQHRRAAMLGAPEVLQLNANIMQAIGAKKVLDIGVFTGASSLSAALALPPNGKVYALDISEEFTNIGKPYWEEAGVSNKISLHIAPAAETLQKFIDAGEAGTFDYAFIDADKESYDRYYELCLILLRPGGVIAFDNTLWDGAVIDPTDQKPGTLAIRKMNEKLKDDQRINISFLRIGDGLSLCFKK

SEQ ID NO: 16 - protein, 363 aa, Arabidopsis thaliana
MGSTAETQLTPVQVTDDEAALFAMQLASASVLPMALKSALELDLLEIMAKNGSPMSPTEIASKLPTKNPEAPVMLDRILRLLTSYSVLTCSNRKLSGDGVERIYGLGPVCKYLTKNEDGVSIAALCLMNQDKVLMESWYHLKDAILDGGIPFNKAYGMSAFEYHGTDPRFNKVFNNGMSNHSTITMKKILETYKGFEGLTSLVDVGGGIGATLKMIVSKYPNLKGINFDLPHVIEDAPSHPGIEHVGGDMFVSVPKGDAIFMKWICHDWSDEHCVKFLKNCYESLPEDGKVILAECILPETPDSSLSTKQVVHVDCIMLAHNPGGKERTEKEFEALAKASGFKGIKVVCDAFGVNLIELLKKL

SEQ ID NO: 17 - protein, 496 aa, Homo sapiens [sequence omitted]

SEQ ID NO: 18 - protein, 448 aa, Homo sapiens
MDDKGNKGSSKREAATESGKTAVVFSLKNEVGGLVKALRLFQEKRVNMVHIESRKSRRRSSEVEIFVDCECGKTEFNELIQLLKFQTTIVTLNPPENIWTEEEELEDVPWFPRKISELDKCSHRVLMYGSELDADHPGFKDNVYRQRRKYFVDVAMGYKYGQPIPRVEYTEEETKTWGVVFRELSKLYPTHACREYLKNFPLLTKYCGYREDNVPQLEDVSMFLKERSGFTVRPVAGYLSPRDFLAGLAYRVFHCTQYIRHGSDPLYTPEPDTCHELLGHVPLLADPKFAQFSQEIGLASLGASDEDVQKLATCYFFTIEFGLCKQEGQLRAYGAGLLSSIGELKHALSDKACVKAFDPKTTCLQECLITTFQEAYFVSESFEEAKEKMRDFAKSITRPFSVYFNPYTQSIEILKDTRSIENVVQDLRINRVHSSALTEKEGVRQPEV

SEQ ID NO: 19 - protein, 428 aa, Homo sapiens
MDDKGNKGSSKREAATESGKTAVVFSLKNEVGGLVKALRLFQEKRVNMVHIESRKSRRRSSEVEIFVDCECGKTEFNELIQLLKFQTTIVTLNPPENIWTEEEELEDVPWFPRKISELDKCSHRVLMYGSELDADHPGFKDNVYRQRRKYFVDVAMGYKYGQPIPRVEYTEEETKTWGVVFRELSKLYPTHACREYLKNFPLLTKYCGYREDNVPQLEDVSMFLKERSGFTVRPVAGYLSPRDFLAGLAYRVFHCTQYIRHGSDPLYTPEPDTCHELLGHVPLLADPKFAQFSQEIGLASLGASDEDVQKLATCYFFTIEFGLCKQEGQLRAYGAGLLSSIGELKHALSDKACVKAFDPKTTCLQECLITTFQEAYFVSESFEEAKEKMRDFAKSITRPFSVYFNPYTQSIEILKDTRSIENVVQDLR

SEQ ID NO: 20 - protein, 315 aa, Homo sapiens
MELEDVPWFPRKISELDKCSHRVLMYGSELDADHPGFKDNVYRQRRKYFVDVAMGYKYGQPIPRVEYTEEETKTWGVVFRELSKLYPTHACREYLKNFPLLTKYCGYREDNVPQLEDVSMFLKERSGFTVRPVAGYLSPRDFLAGLAYRVFHCTQYIRHGSDPLYTPEPDTCHELLGHVPLLADPKFAQFSQEIGLASLGASDEDVQKLATCYFFTIEFGLCKQEGQLRAYGAGLLSSIGELKHALSDKACVKAFDPKTTCLQECLITTFQEAYFVSESFEEAKEKMRDFAKSITRPFSVYFNPYTQSIEILKDT